European Patent Application EP 4 233 897 A1, published August 30, 2023. Title: Vaccine composition for reducing the size or volume of the target tissue comprising genetic material encoding for foreign antigen or Kit. Applicant: SK bioscience Co., Ltd. The sequence listing filed with the application follows.

SEQUENCE LISTING (6 sequences)

SEQ ID NO: 1 - DNA, 2334 bp, Yellow fever virus
atgtctggtcgtaaagctcagggaaaaaccctgggcgtcaatatggtacgacgaggagttcgctccttgtcaaacaaaataaaacaaaaaacaaaacaaattggaaacagacctggaccttcaagaggtgttcaaggatttatctttttctttttgttcaacattttgactggaaaaaagatcacagcccacctaaagaggttgtggaaaatgctggacccaagacaaggcttggctgttctaaggaaagtcaagagagtggtggccagtttgatgagaggattgtcctcaaggaaacgccgttcccatgatgttctgactgtgcaattcctaattttgggaatgctgttgatgacgggtggagtgaccttggtgcggaaaaacagatggttgctcctaaatgtgacatctgaggacctcgggaaaacattctctgtgggcacaggcaactgcacaacaaacattttggaagccaagtactggtgcccagactcaatggaatacaactgtcccaatctcagtccaagagaggagccagatgacattgattgctggtgctatggggtggaaaacgttagagtcgcatatggtaagtgtgactcagcaggcaggtctaggaggtcaagaagggccattgacttgcctacgcatgaaaaccatggtttgaagacccggcaagaaaaatggatgactggaagaatgggtgaaaggcaactccaaaagattgagagatggttcgtgaggaaccccttttttgcagtgacggctctgaccattgcctaccttgtgggaagcaacatgacgcaacgagtcgtgattgccctactggtcttggctgttggtccggcctactcagctcactgcattggaattactgacagggatttcattgagggggtgcatggaggaacttgggtttcagctaccctggagcaagacaagtgtgtcactgttatggcccctgacaagccttcattggacatctcactagagacagtagccattgatagacctgctgaggtgaggaaagtgtgttacaatgcagttctcactcatgtgaagattaatgacaagtgccccagcactggagaggcccacctagctgaagagaacgaaggggacaatgcgtgcaagcgcacttattctgatagaggctggggcaatggctgtggcctatttgggaaagggagcattgtggcatgcgccaaattcacttgtgccaaatccatgagtttgtttgaggttgatcagaccaaaattcagtatgtcatcagagcacaattgcatgtaggggccaagcaggaaaattggaataccgacattaagactctcaagtttgatgccctgtcaggctcccaggaagtcgagttcattgggtatggaaaagctacactggaatgccaggtgcaaactgcggtggactttggtaacagttacatcgctgagatggaaacagagagctggatagtggacagacagtgggcccaggacttgaccctgccatggcagagtggaagtggcggggtgtggagagagatgcatcatcttgtcgaatttgaacctccgcatgccgccactatcagagtactggccctgggaaaccaggaaggctccttgaaaacagctcttactggcgcaatgagggttacaaaggacacaaatgacaacaacctttacaaactacatggtggacatgtttcttgcagagtgaaattgtcagctttgacactcaaggggacatcctacaaaatatgcactgacaaaatgttttttgtcaagaacccaactgacactggccatggcactgttgtgatgcaggtgaaagtgtcaaaaggagccccctgcaggattccagtgatagtagctgatgatcttacagcggcaatcaataaaggcattttggttacagttaaccccatcgcctcaaccaatgatgatgaagtgctgattgaggtgaacccaccttttggagacagctacattatcgttgggagaggagattcacgtctcacttaccagtggcacaaagagggaagctcaataggaaagttgttcactcagaccatgaaaggcgtggaacgcctggccgtcatgggagacaccgcctgggatttcagctccgctggagggttcttcacttcggttgggaaaggaattcatacggtgtttggctctgcctttcaggggctatttggcggcttgaactggataacaaaggtcatcatgggggcggtacttatatgggttggcatcaacacaagaaacatgacaatgtccatgagcatgatcttggtaggagtgatcatgatgtttttgtctctaggagttggggcg

SEQ ID NO: 2 - DNA, 648 bp, Artificial Sequence
  the p35 subunit of interleukin 12
atgtgtcaatcacgctacctcctctttttggccacccttgccctcctaaaccacctcagtttggccagggtcattccagtctctggacctgccaggtgtcttagccagtcccgaaacctgctgaagaccacagatgacatggtgaagacggccagagaaaaactgaaacattattcctgcactgctgaagacatcgatcatgaagacatcacacgggaccaaaccagcacattgaagacctgtttaccactggaactacacaagaacgagagttgcctggctactagagagacttcttccacaacaagagggagctgcctgcccccacagaagacgtctttgatgatgaccctgtgccttggtagcatctatgaggacttgaagatgtaccagacagagttccaggccatcaacgcagcacttcagaatcacaaccatcagcagatcattctagacaagggcatgctggtggccatcgatgagctgatgcagtctctgaatcataatggcgagactctgcgccagaaacctcctgtgggagaagcagacccttacagagtgaaaatgaagctctgcatcctgcttcacgccttcagcacccgcgtcgtgaccatcaacagggtgatgggctatctgagctccgcctga

SEQ ID NO: 3 - DNA, 1008 bp, Artificial Sequence
  the p40 subunit of interleukin 12
atgtgtcctcagaagctaaccatctcctggtttgccatcgttttgctggtgtctccactcatggccatgtgggagctggagaaagacgtttatgttgtagaggtggactggactcccgatgcccctggagaaacagtgaacctcacctgtgacacgcctgaagaagatgacatcacctggacctcagaccagagacatggagtcataggctctggaaagaccctgaccatcactgtcaaagagtttctagatgctggccagtacacctgccacaaaggaggcgagactctgagccactcacatctgctgctccacaagaaggaaaatggaatttggtccactgaaattttaaaaaatttcaaaaacaagactttcctgaagtgtgaagcaccaaattactccggacggttcacgtgctcatggctggtgcaaagaaacatggacttgaagttcaacatcaagagcagtagcagttcccctgactctcgggcagtgacatgtggaatggcgtctctgtctgcagagaaggtcacactggaccaaagggactatgagaagtattcagtgtcctgccaggaggatgtcacctgcccaactgccgaggagaccctgcccattgaactggcgttggaagcacggcagcagaataaatatgagaactacagcaccagcttcttcatcagggacatcatcaaaccagacccgcccaagaacttgcagatgaagcctttgaagaactcacaggtggaggtcagctgggagtaccctgactcctggagcactccccattcctacttctccctcaagttctttgttcgaatccagcgcaagaaagaaaagatgaaggagacagaggaggggtgtaaccagaaaggtgcgttcctcgtagagaagacatctaccgaagtccaatgcaaaggcgggaatgtctgcgtgcaagctcaggatcgctattacaattcctcatgcagcaagtgggcatgtgttccctgcagggtccgatcctag

SEQ ID NO: 4 - DNA, 6 bp, Unknown
  kozak sequence
gccacc

SEQ ID NO: 5 - protein, 1063 aa, Rubella virus
MASTTPITMEDLQKALETQSRALRAELAAGASQSRRPRPPRQRDSSTTGDDSGRDSGGPRRRRGNRGRGQRRDWSRAPPPPEERQETRSQTPAPKPSRAPPQQPQPPRMQTGRGGSAPRPELGPPTNPFQAAVARGLRPPLHDPDTEAPTEACVTSWLWSEGEGAVFYRVDLHFTNLGTPPLDEDGRWDPALMYNPCGPEPPAHVVRAYNQPAGDVRGVWGKGERTYAEQDFRVGGTRWHRLLRMPVRGLDGDSAPLPPHTTERIETRSARHPWRIRFGAPQAFLAGLLLAAVAVGTARAGLQPRADMAAPPTLPQPPRAHGQHYGHHHHQLPFLGHDGHHGGTLRVGQHHRNASDVLPGHWLQGGWGCYNLSDWHQGTHVCHTKHMDFWCVEHDRPPPATPTPLTTAANSTTAATPATAPAPCHAGLNDSCGGFLSGCGPMRLRHGADTRCGRLICGLSTTAQYPPTRFGCAMRWGLPPWELVVLTARPEDGWTCRGVPAHPGTRCPELVSPMGRATCSPASALWLATANALSLDHALAAFVLLVPWVLIFMVCRRTCRRRGAAAALTAVVLQGYNPPAYGEEAFTYLCTAPGCATQAPVPVRLAGVRFESKIVDGGCFAPWDLEATGACICEIPTDVSCEGLGAWVPTAPCARIWNGTQRACTFWAVNAYSSGGYAQLASYFNPGGSYYKQYHPTACEVEPAFGHSDAACWGFPTDTVMSVFALASYVQHPHKTVRVKFHTETRTVWQLSVAGVSCNVTTEHPFCNTPHGQLEVQVPPDPGDLVEYIMNHTGNQQSRWGLGSPNCHGPDWASPVCQRHSPDCSRLVGATPERPRLRLVDADDPLLRTAPGPGEVWVTPVIGSQARKCGLHIRAGPYGHATVEMPEWIHAHTTSDPWHPPGPLGLKFKTVRPVALPRTLAPPRNVRVTGCYQCGTPALVEGLAPGGGNCHLTVNGEDLGAFPPGKFVTAALLNTPPPYQVSCGGESDRASARVIDPAAQSFTGVVYGTHTTAVSETRQTWAEWAAAHWWQLTLGAICALLLAGLLACCAKCLYYLRGAIAPR

SEQ ID NO: 6 - protein, 623 aa, Unknown
  the gE protein of the Varicella zoster virus
MGTVNKPVVGVLMGFGIITGTLRITNPVRASVLRYDDFHIDEDKLDTNSVYEPYYHSDHAESSWVNRGESSRKAYDHNSPYIWPRNDYDGFLENAHEHHGVYNQGRGIDSGERLMQPTQMSAQEDLGDDTGIHVIPTLNGDDRHKIVNVDQRQYGDVFKGDLNPKPQGQRLIEVSVEENHPFTLRAPIQRIYGVRYTETWSFLPSLTCTGDAAPAIQHICLKHTTCFQDVVVDVDCAENTKEDQLAEISYRFQGKKEADQPWIVVNTSTLFDELELDPPEIEPGVLKVLRTEKQYLGVYIWNMRGSDGTSTYATFLVTWKGDEKTRNPTPAVTPQPRGAEFHMWNYHSHVFSVGDTFSLAMHLQYKIHEAPFDLLLEWLYVPIDPTCQPMRLYSTCLYHPNAPQCLSHMNSGCTFTSPHLAQRVASTVYQNCEHADNYTAYCLGISHMEPSFGLILHDGGTTLKFVDTPESLSGLYVFVVYFNGHVEAVAYTVVSTVDHFVNAIEERGFPPTAGQPPATTKPKEITPVNPGTSPLLRYAAWTGGLAAVVLLCLVIFLICTAKRMRVKAYRVDKSPYNQSMYYAGLPVDDFEDSESTDTEEEFGNAIGGSHGGSSYTVYIDKTR